European Patent Specification EP 3 654 032 B1, published September 27, 2023. Title: Disease detection method. Applicant: Shimadzu Corporation. The sequence listing filed with the application follows.

SEQUENCE LISTING (14 sequences)

SEQ ID NO: 1 - protein, 17 aa, Homo sapiens
APLQPVTPLQLFEGRRN

SEQ ID NO: 2 - protein, 16 aa, Homo sapiens
PGRQSQEGAGLPSHHG

SEQ ID NO: 3 - protein, 11 aa, Homo sapiens
AAPPGAEGNRT

SEQ ID NO: 4 - protein, 17 aa, Homo sapiens
KLAELPAAAQPSAEDSD

SEQ ID NO: 5 - protein, 21 aa, Homo sapiens
TATSEYQTFFNPRTFGSGEAD

SEQ ID NO: 6 - protein, 14 aa, Homo sapiens
APVIHQEMIGGLRN

SEQ ID NO: 7 - protein, 16 aa, Homo sapiens
QTASGQALKGDGGLYS

SEQ ID NO: 8 - protein, 20 aa, Homo sapiens
GLGLSYLSSHIANVERVPFD

SEQ ID NO: 9 - protein, 14 aa, Homo sapiens
RSGGNATLQVDSWP

SEQ ID NO: 10 - protein, 19 aa, Homo sapiens
NIAIVGDVRLVGEVPSSGT

SEQ ID NO: 11 - protein, 13 aa, Homo sapiens
TATSEYQTFFNPR

SEQ ID NO: 12 - protein, 12 aa, Homo sapiens
GLDEDSDRAIEG

SEQ ID NO: 13 - protein, 13 aa, Homo sapiens
GLDEDSDRAIEGR

SEQ ID NO: 14 - protein, 14 aa, Homo sapiens
GVSGSHFVGVDGVR